European Patent Specification EP 3 793 347 B1, published October 1, 2025. Title: A SOLANACEAE PLANT RICH IN ANTHOCYANINS CONCENTRATION. Applicant: ENZA ZADEN BEHEER B.V. The sequence listing filed with the application follows.

SEQUENCE LISTING (18 sequences)

SEQ ID NO: 1 - DNA, 2217 bp, Capsicum annuum
atgggtgaactttcaagccaagaacctcttcttttaaagaaagaaaatgaatttaattatctcaagaagatacctcttttggtatcatcaacaatcaaaggaataatgtgggtgatcttcattgcatgggcagcttttttctttgtgttgcctacagaatttggaagagaattgcaacataaaactataagagccacaaatggaactctttttgggactacaggaagcacattcttgttattcagtttcccagttttcatgattgcatttcttggaattattcgtctcgttctctctggtgaagatgaacctcaagtcaagaagactgcaaaaggtccaaagtttagattgtggacattcccggtgctggtggatggaccatttggtgttgttacagctacagaaatgattggtgttatactcttctcagtgtacatcgtgtgggctgtaataatgtacactatacagaatgttgacctcttatccttgtttgatgcacacggcatgaaagagaaaagtgctttgttgctggagctgacaggccttcgttttggattcattggattaatctgcttagcatttttgtttctgcctgttgcacgaggttcagttcttcttcgagctatagatatcccttttgaacatgccactagatatcatgtttggctgggacatcttactatggctctttttactcttcatggtctgttctatgtgattggctgggcaatgcggggacgacttgtggaagaactagttgactggaaaaacgtaggagtggccaatcttccaggagttatcagccttgcagctggtttactgatgtgggtgacttcacttcctggattaaggagaaaaaactttgaactgttcttctatacacaccaattgtatgtggtgttcgtggtattcctggtcttgcatgttggtgatttcatcttcatgatggctggagctgggatcttcctgttcatgcttgatcggttccttagattcttccagtcaagaaagactgttgacatactttcagccacatgtttcccttgtggaaccgttgaactcgttatctcaaaacctgcaaatttagattacaacgcccttggctggatattcttacaaatacgcgagttgtcctggctgcagtggcaccctttcagtgtctcatctagtccccttgatgggaaacagcatcttgctattctgataaaggttcttggagattggacagagaaactgaagggaaacatcttgaatctttctgtagagcaatctgagacggagccgcttttgcagcataacaggaaaataacagcttctgttgaaggtccttatggacatgaatcaccataccacttaacgtatgaaaatctcattttggtagcaggtggaattggaatttctccctttctagctatcctgagtgatattctccaccatatcaatgatggcaagccttgtctgtcaagaaatatactgatagtatgggctatcaaaaattcggacgagcttccacttcttgatacagttgacatggaggcaatctgtccacttttctctgataaactgaatcttgagcttcaaacatttgtgactcgggaatcacagcctccattggaggagggtaaaacacccaaagcaatgcaaccctcaatctcccctggcttcaagggatgccgaatgtctggtttggttggtactggaaatattgtatggtctggattatatgtcgtagtatccaccatagggttggtgatcactacagcgtcgctgaacattttctacgtaaatccattcaatgtatattattggtggtacaaagggcttttgttgattggatgcatggctgcaagcattcttatatttggtggtctcgtgatcgctttatggcatctttgggaaaggaaaacctcatcgaaggaggaaccagaggacgacacaaagaaagttgacatcctgcagcaccagaatgaagcctctttacccaagagttttggagaggctcgatttgtcaacaatattcgatatggtcaaagaccggatttccaagagatatttggatcgcatgcaaagagctggggaagtgtagatattggtgtgattgtgtgtggtcctcctactcttcagactagtgttgctaaagagtgcagaaggcagaacttgcagagaagaggccatcaggctattttccatttcaacagccacagttttgacctctag

SEQ ID NO: 2 - protein, 738 aa, Capsicum annuum
MGELSSQEPLLLKKENEFNYLKKIPLLVSSTIKGIMWVIFIAWAAFFFVLPTEFGRELQHKTIRATNGTLFGTTGSTFLLFSFPVFMIAFLGIIRLVLSGEDEPQVKKTAKGPKFRLWTFPVLVDGPFGVVTATEMIGVILFSVYIVWAVIMYTIQNVDLLSLFDAHGMKEKSALLLELTGLRFGFIGLICLAFLFLPVARGSVLLRAIDIPFEHATRYHVWLGHLTMALFTLHGLFYVIGWAMRGRLVEELVDWKNVGVANLPGVISLAAGLLMWVTSLPGLRRKNFELFFYTHQLYVVFVVFLVLHVGDFIFMMAGAGIFLFMLDRFLRFFQSRKTVDILSATCFPCGTVELVISKPANLDYNALGWIFLQIRELSWLQWHPFSVSSSPLDGKQHLAILIKVLGDWTEKLKGNILNLSVEQSETEPLLQHNRKITASVEGPYGHESPYHLTYENLILVAGGIGISPFLAILSDILHHINDGKPCLSRNILIVWAIKNSDELPLLDTVDMEAICPLFSDKLNLELQTFVTRESQPPLEEGKTPKAMQPSISPGFKGCRMSGLVGTGNIVWSGLYVVVSTIGLVITTASLNIFYVNPFNVYYWWYKGLLLIGCMAASILIFGGLVIALWHLWERKTSSKEEPEDDTKKVDILQHQNEASLPKSFGEARFVNNIRYGQRPDFQEIFGSHAKSWGSVDIGVIVCGPPTLQTSVAKECRRQNLQRRGHQAIFHFNSHSFDL

SEQ ID NO: 3 - DNA, 2223 bp, Solanum lycopersicum
atgggtgaactctcaagccaagaacctcttcttttgaaaaaagaaaatgaatttgattctctcagaaagacaccatttttaatctcatcaacaaagttgattctcaaagtattaatgtgggtgatttttatttcatgggctgcttttattttcttgttgccaacaaagttcactaatgaaatttttgggacaattgttggagccaccaaaggatctatttttcggacagcaggtagcacatccttgttattcagtttcccaattatcatgattgcatttcttgcaattattcttctcgttgtctcgggtgaagatcaacctcaaatcaagaaggctggtaaaggaccaacttttagattatggacattccctgtgctggtggatggaccatttggggttgttacagctgcggaaatgattggcgttataatcttctcggtctacatcgtctgggctgtagttatgtatagtatacagaatgttgacatcttatctttgtatcatttaccagacatgaaagagagaagtgctaagttgctggagctgacaggtctccgttttggattcattggattaatctgcttagcgtttttgtttctgcctgttgcacgtggttcagttcttcttcgagccatagatatcccttttgaacatgccactagatatcatgtttggctgggacatcttactatggctatttttagccttcatggtctattctatattattggctgggcaattcaagggagacttttggaagaactagtcggctggaaaaacataggaatagccaatcttccaggagttatcagccttttagctggtttattgatgtggttgacttcacttcctggagtaaggagaaaaaactttgagctgttcttctatacacaccaattgtatgtggtgtttgtggtgttcctggctttgcatgttggtgatttcgtcttcatgatggctggagctgggatcttcctgttcatgcttgatcggttccttagattcttccagtcacgaaagacagttgacatactttcggccacatgctttccttgtggaaccgttgaactcgttatttcaaaacctgcaaatttacattacaacgctcttggctggatattcttacaaatacgcgagttgtcctggctgcagtggcaccctttcagtgtctcttctagtccccttgatggcaaacatcatcttgcgattctcataaaggttcttggagattggactgaaaaactgaagggaaacatcttgaatctttctgtagaagaatctgagacggagcctcttttgctgcataacaggaaaattacagcttctgttgaaggtccttatggacatgaatcaccataccacttaacgtatgaaaatctcattttggtagcaggtggaattggaatttctcccttcctagctatcctgagtgatatcctccaccgtatcaacgatagctcgccttgcctgccaagaaatatactaatagtatgggctatcaaaaactcagatgagcttccacttcttgaaacagttgacatggaggcaatctgtccacttttctctgataaactgaatcttgagattcaaacatatgtgacacgggaatcacagccttcattggaggagggtaaaacacccaaagcaatgcaccactcaatctcccctggcttcaaaggatgtcgaatgtctggtttggttggtactggacatgtcgtatggtctggattatatgtcatagtatccaccatagggtttgtgatcactgtagcattgctggacattttctacataaatccattcaatataacttactggtggtacaaggggcttttgttgattggatgcatgactgcaagtattcttatatttgggggtttcgttatcgctttatggcatctttgggagaggaaaacctcatcgaaggaggaaccacaggacgccacaaagaaagctgacatcttgcagcagaatgaagcctctttagacagtaactttggagaggctcgatatgttaataatattcgatatggtcaaagacctgatttccaagagatatttggatcacatgcaaagagctggggaagtgtagatattggtgtaattgtgtgtggtcctcctactcttcagtccagtattgctaaagaatgcagaagccagaacttgaagagaagaggtcgtcaggctattttccatttcaacagccacagttttgacctctag

SEQ ID NO: 4 - protein, 740 aa, Solanum lycopersicum
MGELSSQEPLLLKKENEFDSLRKTPFLISSTKLILKVLMWVIFISWAAFIFLLPTKFTNEIFGTIVGATKGSIFRTAGSTSLLFSFPIIMIAFLAIILLVVSGEDQPQIKKAGKGPTFRLWTFPVLVDGPFGVVTAAEMIGVIIFSVYIVWAVVMYSIQNVDILSLYHLPDMKERSAKLLELTGLRFGFIGLICLAFLFLPVARGSVLLRAIDIPFEHATRYHVWLGHLTMAIFSLHGLFYIIGWAIQGRLLEELVGWKNIGIANLPGVISLLAGLLMWLTSLPGVRRKNFELFFYTHQLYVVFVVFLALHVGDFVFMMAGAGIFLFMLDRFLRFFQSRKTVDILSATCFPCGTVELVISKPANLHYNALGWIFLQIRELSWLQWHPFSVSSSPLDGKHHLAILIKVLGDWTEKLKGNILNLSVEESETEPLLLHNRKITASVEGPYGHESPYHLTYENLILVAGGIGISPFLAILSDILHRINDSSPCLPRNILIVWAIKNSDELPLLETVDMEAICPLFSDKLNLEIQTYVTRESQPSLEEGKTPKAMHHSISPGFKGCRMSGLVGTGHVVWSGLYVIVSTIGFVITVALLDIFYINPFNITYWWYKGLLLIGCMTASILIFGGFVIALWHLWERKTSSKEEPQDATKKADILQQNEASLDSNFGEARYVNNIRYGQRPDFQEIFGSHAKSWGSVDIGVIVCGPPTLQSSIAKECRSQNLKRRGRQAIFHFNSHSFDL

SEQ ID NO: 5 - DNA, 2229 bp, Solanum melongena
atgggtgaactctcaggccaagaacctttacttttgaaaaaagaagaatttaattatctcaacaagacaccactttgggtgtcatcaacaaagttgattctcaatgtagtaatttgggtgactttcattgcctgggcagcttttattttcttcttgccaacagaattcactaatgaactggaagggaaaattattaaagccaccaaaggaactatttttgggactacaggaagcacattcttgatcttcagtttcccaattttcttgattgcatttcttgcaattattcgtctcattctctcgggtgaagaaccccaaatcaagaaggctgcaaaaggtccaagatttagattatggacattcccagtgctggtggatggaccatttggtgttgttacagctgcggaaatgattggcgttgtactcttctcagtgtacatcgtttgggctgtagttatgtatactataaaggatattgacctcttatccttgtttcatccaagagacatgaaagagagaagtgctctgtttctggaggtaacaggcctccgttttggattcattggattaatctgcttagcatttttgtttctgcctgttgcacgtggttcagttcttcttcgagctatagatatcccttttgaacatgccactagatatcatgtttggctgggacatctcactatggctctttttagcctccatggtctgttctatatgattggctgggcaatgcaaggccgacttgcggaagaactagccagctggaaaaacgtaggaatagccaatcttccaggagtgatcagccttgcagctggtttattgatgtgggtgacttcacttcccggattaaggagaaaaaactttgaactgttcttctatacgcatcaattgtatgtggtgttcgtggtgttcctggccttgcatgttggtgatttcatcttcatgatggctggagctgggatcttcctgttcatgcttgatcggttccttagattcttccagtcacgaaagacagtggacatactttcagccaaatgctttccttgtggaactgtcgaacttgttatttccaaacctgcaaatttacattacaactcccttggctggatattcttacaaatacgcgagttgtcctggctacagtggcaccctttcagtgtctcctctagtccacttgatgggaaacatcatcttgcaattctcataaaggttctaggagattggaccgaaaaactgaagggaaacatcttaaacctttctgtagaagaatctgagacgaagcctcttttgcatcataacaggaaaataacagcttctgttgaaggtccttatggtcatgaatcaccataccacttaacgtataaaaatctcattttggtagcaggtggaattggaatttctcccttcctagctatcctgagtgatattctccaccgtatcaatgatagcactccttgtctgccaagaaatatactaatagtatgggctatcaaaaattcagatgagcttccacttctcgagacagttgacatggaggcaatctgtccacttttctctgataaactgaatcttgaaattcaaacatttgtgacacgggaatcacagccttcattggaggagggtaaaacacccaaagcaatgcaaaccccgtcaatctgccctggcttcaagggatgtcaaatgtctggtttggttggtactggaaatgttgtatggtctggattatatgtcatagtatccaccatagggttggtgatcactgtagcgttgctggacatttactacataaatccattcaatgtaacttactggtggtacaagggacttttgttgattggatgcatgactgcaagtattcttatatttgggggtttcgttatcattttatggcatctttgggaaaggaaagccccatcgaaggaggaaccagaggatgccacacagatagttgacgttttgcagcagcagcagcagaatgaagcctctttacccaagagttctggagaggctcgatatgttaataatattcgatatggtcaaagaccagatttccaagagatatttggatcacatgcaaagagttggggaagtgtagatataggtgtgattgtgtgtggtcctcctactcttcaatccagtgttgctaaagagtgcagaagtcagaacttgcagagaagaggccatcaggctattttccacttcaacagccacagttttgacctctag

SEQ ID NO: 6 - protein, 742 aa, Solanum melongena
MGELSGQEPLLLKKEEFNYLNKTPLWVSSTKLILNVVIWVTFIAWAAFIFFLPTEFTNELEGKIIKATKGTIFGTTGSTFLIFSFPIFLIAFLAIIRLILSGEEPQIKKAAKGPRFRLWTFPVLVDGPFGVVTAAEMIGVVLFSVYIVWAVVMYTIKDIDLLSLFHPRDMKERSALFLEVTGLRFGFIGLICLAFLFLPVARGSVLLRAIDIPFEHATRYHVWLGHLTMALFSLHGLFYMIGWAMQGRLAEELASWKNVGIANLPGVISLAAGLLMWVTSLPGLRRKNFELFFYTHQLYVVFVVFLALHVGDFIFMMAGAGIFLFMLDRFLRFFQSRKTVDILSAKCFPCGTVELVISKPANLHYNSLGWIFLQIRELSWLQWHPFSVSSSPLDGKHHLAILIKVLGDWTEKLKGNILNLSVEESETKPLLHHNRKITASVEGPYGHESPYHLTYKNLILVAGGIGISPFLAILSDILHRINDSTPCLPRNILIVWAIKNSDELPLLETVDMEAICPLFSDKLNLEIQTFVTRESQPSLEEGKTPKAMQTPSICPGFKGCQMSGLVGTGNVVWSGLYVIVSTIGLVITVALLDIYYINPFNVTYWWYKGLLLIGCMTASILIFGGFVIILWHLWERKAPSKEEPEDATQIVDVLQQQQQNEASLPKSSGEARYVNNIRYGQRPDFQEIFGSHAKSWGSVDIGVIVCGPPTLQSSVAKECRSQNLQRRGHQAIFHFNSHSFDL

SEQ ID NO: 7 - DNA, 2106 bp, Petunia axillaris
  1
atggggctttttgtggttgtcatgtcaaccaacctgaggaaagccattgccttgttcaaagtcccaggcacgattactgctactaatgcgagaatggcgagctgcattggttactgtggaagcacattcttgattttctgtttcccaatcttcatgattgcatttcttgccattattcatctgagtctctctagtgaagatgaaccacaagtgaagaaaacctcaaaaggtccacgttttcgcttgtggacattcccagttttggttgatggaccactaggggttgtgacagctgcagaaattattggaattatactcttctgtgtgtatatcatctgggctgttattgtgtatagtattcaaaacatcaacaccttatactcatctgatgtacatactgtgaaagagaaaagtgctttgatgctggagctcacaggtcttcactttggatccattggattaatctgcttagcatttttgtttctgcccgttgcaaggggttcagttcttcttcgagctgtagatatcccttttgagcacgcaacaagatatcatgtttggctgggacatctaacaatgcttctttttactcttcatggtctatcctacttgattagctgggcaatgcaggggcgtcttgtacatgaaataatggatttgaacagtacagaagttgtcaatcttccaggagttatcagcctagcagctggtttattgatgtgggtgacatcacttcctggagttaggagaagaaacttcgaactattcttctatacgcaccaactgtacataatattcgttttattcctggccttgcatgttggtgatttcatcttcatgactgctggtgctggaatattccttttcatgcttgatcgcttccttagattctgtcagtcgcgatggactgttgacatactttcagctacatgctttcctaatggaactgttgaagttgttctttcaaaacctgcaaatcttcactacagtgcccttagttgggtatttcttcaagttcgtgaattatcctggctgcaatggcacccttttagtgtctcgtcaagtcctcttgatggaaaacatcatctttcagtcctcataaaagtactaggagactggaccgaaaagctgaagggacatgtcttggatctttctgtagaacaacctcaaatggagcacctcttgcagaatcattgcaagataactgcttctgttgaagggccttatgggcatcaatctccatatcatttgacgtatgaaaaccttattttggtggcaggcggcataggaatttcccctttcctagctatcttgagcgatattctccaccggattaatgacagcaagccttgtctgccaagaaatattttaatagtgtgggccgtgaaaaaatcagatgagcttccacttcttgagacaattgacatggaggcaatatgtccatttttctgtgataaactgaatcttgagattcaaacatttgttactcgagaagcacaaccttcattggaggagggtacaacactcaagggtgtaaatccctctgtttcccctagcctcaagggatgtccaatgtctggtttggttggtacaggaaatgttatatggtctggaatttatgtccttgtttccataattggcatggtgatcactgtggcattgctagacatttattacgtaaatccattacattacgggtggtaccatgggcttctgttaattggatgtatggttgctagtattgttacctttggaggtcttgtcattggtttatggcatctttgggaaaagaaaacctcagtgcaagttgaagcagaggataccaagaaggttaacattctgcaggagtgtgaggctggcctaaacaagctttccaatcttgtcgaggctcagtctgctaatactatccaatatggtgaaagaccaaattttaaagatatatttggatcatatgcagagagctggggaagcgttgatattggtgtaatcgtgtgtggtcctcctaccctccagtctaccgttgctaaagagtgcagaagacagaacttgaagagaagtggtaatcaggctatattccatttcaacagccatagttttgacctatag

SEQ ID NO: 8 - protein, 701 aa, Petunia axillaris
  1
MGLFVVVMSTNLRKAIALFKVPGTITATNARMASCIGYCGSTFLIFCFPIFMIAFLAIIHLSLSSEDEPQVKKTSKGPRFRLWTFPVLVDGPLGVVTAAEIIGIILFCVYIIWAVIVYSIQNINTLYSSDVHTVKEKSALMLELTGLHFGSIGLICLAFLFLPVARGSVLLRAVDIPFEHATRYHVWLGHLTMLLFTLHGLSYLISWAMQGRLVHEIMDLNSTEVVNLPGVISLAAGLLMWVTSLPGVRRRNFELFFYTHQLYIIFVLFLALHVGDFIFMTAGAGIFLFMLDRFLRFCQSRWTVDILSATCFPNGTVEVVLSKPANLHYSALSWVFLQVRELSWLQWHPFSVSSSPLDGKHHLSVLIKVLGDWTEKLKGHVLDLSVEQPQMEHLLQNHCKITASVEGPYGHQSPYHLTYENLILVAGGIGISPFLAILSDILHRINDSKPCLPRNILIVWAVKKSDELPLLETIDMEAICPFFCDKLNLEIQTFVTREAQPSLEEGTTLKGVNPSVSPSLKGCPMSGLVGTGNVIWSGIYVLVSIIGMVITVALLDIYYVNPLHYGWYHGLLLIGCMVASIVTFGGLVIGLWHLWEKKTSVQVEAEDTKKVNILQECEAGLNKLSNLVEAQSANTIQYGERPNFKDIFGSYAESWGSVDIGVIVCGPPTLQSTVAKECRRQNLKRSGNQAIFHFNSHSFDL

SEQ ID NO: 9 - DNA, 2220 bp, Petunia axillaris
  2
atgggtgaatattcaggccaagaacctcttcttttgaagaaagaagatgacttcaactatctcaagaagacacccttttgggtatcatcaacaaagttaattctcaaagtagtaatgtggatgatcttcattgcatgggcaacttttcttttcttattgcctgcaaatttcatggctgaattgcaagggatatgtgttcgagctaccaaggaaactatttttggaactactggaagcatattcttgatatacagtttcccaattctaataattgcgtttcttgcaattattcgtcttgttctcactggtgaagatgagcctacagtgaagaagactacaaaaggaccaagttttcggttgtggacatttcctgttttggtggatggaccatttggggttgttacagctgcagaaattattggagttatactcttctcagtgtacataatctgggctgttattatgtacactatacggaatattgacaccttatccgggtttcacgtagaggagacgaatagaagtgctctgttccttgatctaactggccttcgttttggattcattggattagtgtgcttagcatttttgtttctgcctgttgcacggggttcagttcttcttcgagctatagatatcccctttgaacatgccactagatatcatgtttggttgggacatcttacgatggctctttttagccttcatggtctctgctatgtgattagttgggcaatgcgagggcgccttatagaggagctacttgagtggaaaagcataggaatagccaatcttcctggagttatcagccttgcagctggtttattgatgtgggtgacatcacttcctggtgtaaggagaaaaaactttgaattgttcttctatacacaccaattatatgtggtgttcgtggtgttctttgccttgcatgttggcgacttcatcttcatgatagctggtgctggaatcttcctgttcatgcttgatcggttccttagattctggcagtcgcggaagactgttgacatactttcagccacatgttttccttgtggaaccgttgagattgttctttcaaaacctgcaaatttacattacaacgcccttggctggatatttttacaaatacgcgagttatcctggctgcagtggcaccctttcagtgtctcctctagtccccttgatgggaaacatcatattgcaattctcataaaggttcttggagattggactgagaaactgaaggggcgtatcttgaatctctctgttgagcaatctgagatggagccccttttgcagcataacagcaaaataactgcatctgttgaaggtccttatggccatgaatcgccgtatcatttaacgtatgaaaatctcattctggtggcaggtggaataggaatttcccctttcctagctatcctaagtgatatcctccaccgaatcaatgatagcagaccttgcttgccaagaaatgtactaatagtgtgggctataaaaaagacagatgagcttccacttcttgagactgttgacatgcaggcaatctgtccacttttctctgataaactgaatctggagattcaaacatttgtgactcgagaatctcagccttcgctggaggaggggaaaacacccaaagtaatgcacccctcaatctgtcctggcttcaagggatgtcaaatgtctagtttggttggtactggaaatgttgtatggtctggaatatatgtcatagcatccaccattgggttggtaatcactgtagcattgctgaacattttctacgtaaatccattcaatgtatattactggtggtacaaggggcttttgttgattggatgcatggctgcaagtgttgttatttttgggggtctagtgattgccttatggcatctttgggagaggaaaacgtctttgaaggaggaaccagaggacgccaacaagaaagttgacatcctgcagcaaaatgaggccgatttacagaacaatcttgaacaagctcgatttgtcaataatgttcgatacggtcaaagaccagatttccaagaaatatttggatcacatgcaaagagttggggaagtgtagatattggtgtcatagtgtgtggtcctcctactcttcagaccactgtggctaaagagtgcagaagacagaacttgcaaagaagagggcatgaggcaattttccatttcaacagccacagttttgacctctag

SEQ ID NO: 10 - protein, 739 aa, Petunia axillaris
  2
MGEYSGQEPLLLKKEDDFNYLKKTPFWVSSTKLILKVVMWMIFIAWATFLFLLPANFMAELQGICVRATKETIFGTTGSIFLIYSFPILIIAFLAIIRLVLTGEDEPTVKKTTKGPSFRLWTFPVLVDGPFGVVTAAEIIGVILFSVYIIWAVIMYTIRNIDTLSGFHVEETNRSALFLDLTGLRFGFIGLVCLAFLFLPVARGSVLLRAIDIPFEHATRYHVWLGHLTMALFSLHGLCYVISWAMRGRLIEELLEWKSIGIANLPGVISLAAGLLMWVTSLPGVRRKNFELFFYTHQLYVVFVVFFALHVGDFIFMIAGAGIFLFMLDRFLRFWQSRKTVDILSATCFPCGTVEIVLSKPANLHYNALGWIFLQIRELSWLQWHPFSVSSSPLDGKHHIAILIKVLGDWTEKLKGRILNLSVEQSEMEPLLQHNSKITASVEGPYGHESPYHLTYENLILVAGGIGISPFLAILSDILHRINDSRPCLPRNVLIVWAIKKTDELPLLETVDMQAICPLFSDKLNLEIQTFVTRESQPSLEEGKTPKVMHPSICPGFKGCQMSSLVGTGNVVWSGIYVIASTIGLVITVALLNIFYVNPFNVYYWWYKGLLLIGCMAASVVIFGGLVIALWHLWERKTSLKEEPEDANKKVDILQQNEADLQNNLEQARFVNNVRYGQRPDFQEIFGSHAKSWGSVDIGVIVCGPPTLQTTVAKECRRQNLQRRGHEAIFHFNSHSFDL

SEQ ID NO: 11 - DNA, 2211 bp, Petunia axillaris
  3
atgggtgaatattcaggccaagaacctcttcttttgaagaaagaagatgacttcaactacctcaagaagacaccattttggataccatcaacaaagttaattctcaaagtagtaatgtgggtgattttcattgcatgggcaacttttcttttcttattgcctacaaatttcatgaaagaattgcaagagaaatgtattgaagccaccaatggaactatttttggggaaactggaagcatattcttgatgttcagtttcccaattcttataattgcattccttgcaattattcgtctcgctctgagtactggtgaagatgaacctctagtgaagaagacagcaaaaggtccaaattttcgcttatggacatttccagttttggtggatggaccattaggggttgttacagctgcagaaatgattggaattattgtcttctcggtgtacataatctgcgctgttattatgtacactatacggaatattgatgcactatcctggtttcatttagaggaaacgaatagaagtgctctatttctgcagctaacaggccgtcatttgggatccatgggattagtctgcttaggatttttgtttctaccagttgcacggggttcagttcttcttcgagctatagatataccttttgaacatgccattagatatcatgtttggctgggacatcttactatggctctttttagccttcatggtctgttctatgtgattggctgggcaatgcgggggcgccttgtggaaatggtgagcgtaggagtagcccatcttccaggagttatcagccttgcagctggtttagtgatgtgggtgacatcacttcctggtgtaaggagaaaaaactttgaattgttcttctatacacaccaactatatgtagtattcgtggtattcctcgccttgcatgttggtgacttcacttttgtgatagctggtgctgggatcttcctgttcatgcttgatcggttccttagattctgccagtcacggaggacagttgacattctttcagccacatgtttaccttgtggaaccattgaagttgttcttccaaaacctgcaaatttacattacaacgcccttggctggatatttttacagatacgcgagttatccttgctgcagtggcaccctttcagtgtctcctctagtcctcttgatggaaaacatcatattgcaattctcataaagggtcttggagattggactgagaaactgaagggacgtatcttgaatctctctgtagagcaatttgagatggagccccttttgcagcataacagcaaaataacagcttctgttgaaggtccttatggccatgaatcaccatatcatttaacgtatgaacatctcattttggtagcaggcggaattggaatttcccctttcctagccatcctgagcgatatcctccaccgtatcaatgatagcagaccttgcttgccaagaaatatactaatagtatgggctataaaaaagacagatgagcttccacttcttgagacactagacatggaggcaatctgtccacttttctctgataaactgaatctggagattcaaacatttgtcactcgagaatctcaaccttccgtggaggagggtaaaacacccaatgcaatgaacacctcaatctgcccaggcttcaaaggatgtcaaatgtctagtttgattggtactggaaatgttatatggtctggattatatgtcattgtatccacaattgggttggtgatcactgtagctttactgaacatcttctacataaatcctttcaatgtacattactggtggtacaaggggcttttgttgatcggatgcatggctgcaagtattcttatatttgggggtccagtgatcgctttatggcatttttgggaaaggaaaaccttattgaaggaggaatcagaggatgtcaaaaagaaggttgacatccagcagcagaatgaggctagtttacaaaagaatcttggggaggctcgatatgtcaataatattcgatatggtgaaagacctgatttccaagaaatatttggattacatgcaaagagttggggaagtgtagatattggtgtcatagtgtgtggtcctcctactcttcagtccagtgttgctaaagagtgcagaaggcagaacttgcaaagaagagggcatgaggccattttccattttaacagccacagttttgacctctag

SEQ ID NO: 12 - protein, 736 aa, Petunia axillaris
  3
MGEYSGQEPLLLKKEDDFNYLKKTPFWIPSTKLILKVVMWVIFIAWATFLFLLPTNFMKELQEKCIEATNGTIFGETGSIFLMFSFPILIIAFLAIIRLALSTGEDEPLVKKTAKGPNFRLWTFPVLVDGPLGVVTAAEMIGIIVFSVYIICAVIMYTIRNIDALSWFHLEETNRSALFLQLTGRHLGSMGLVCLGFLFLPVARGSVLLRAIDIPFEHAIRYHVWLGHLTMALFSLHGLFYVIGWAMRGRLVEMVSVGVAHLPGVISLAAGLVMWVTSLPGVRRKNFELFFYTHQLYVVFVVFLALHVGDFTFVIAGAGIFLFMLDRFLRFCQSRRTVDILSATCLPCGTIEVVLPKPANLHYNALGWIFLQIRELSLLQWHPFSVSSSPLDGKHHIAILIKGLGDWTEKLKGRILNLSVEQFEMEPLLQHNSKITASVEGPYGHESPYHLTYEHLILVAGGIGISPFLAILSDILHRINDSRPCLPRNILIVWAIKKTDELPLLETLDMEAICPLFSDKLNLEIQTFVTRESQPSVEEGKTPNAMNTSICPGFKGCQMSSLIGTGNVIWSGLYVIVSTIGLVITVALLNIFYINPFNVHYWWYKGLLLIGCMAASILIFGGPVIALWHFWERKTLLKEESEDVKKKVDIQQQNEASLQKNLGEARYVNNIRYGERPDFQEIFGLHAKSWGSVDIGVIVCGPPTLQSSVAKECRRQNLQRRGHEAIFHFNSHSFDL

SEQ ID NO: 13 - DNA, 522 bp, Capsicum annuum
atgagcaaacctggttgtgataacaaagaggaaatgcataaaggatcttggtctaaacaagaagatcaaaaactcattgattatatcactaaacatggtgaaggttgttggagagatttacctaaagctgctggtctacttcgttgcggaaaaagttgtaggctaagatggatgaattatcttaacccaaatttaaaaagaggaaatttttctgaggatgaagatgatctcatcatcaagcttcatgctcttcttggcaataggtggtccttaatagctggaagattgccaggaagaactgataatgaagtgaagaattattggaattcccatttgagaagaaaacttataaaaatgggaatcgatccaaaaaatcataatatttctcattatcttcgtataaaaagacttgaatatttccaagaaaatggcataaaatcagaaaataatgcagtaatatctgatgctacaagttctaattgtgttacaagttcattgcctgatcttaattcacttccatag

SEQ ID NO: 14 - protein, 173 aa, Capsicum annuum
MSKPGCDNKEEMHKGSWSKQEDQKLIDYITKHGEGCWRDLPKAAGLLRCGKSCRLRWMNYLNPNLKRGNFSEDEDDLIIKLHALLGNRWSLIAGRLPGRTDNEVKNYWNSHLRRKLIKMGIDPKNHNISHYLRIKRLEYFQENGIKSENNAVISDATSSNCVTSSLPDLNSLP

SEQ ID NO: 15 - DNA, 537 bp, Solanum lycopersicum
atgagaaagccttgttgtgataacaaagaagaaatgcataaaggagcttggtctaaacaagaagatcaaaaactcattgattatatcactaaacatggtgaaggttgctggagaaatttacctaaagctgctggcctgcttcgttgtggaaaaagttgtaggctaagatggatgaattatcttaatccaaatctaaaaagaggaaatttttctgaggatgaagatgatctaatcatcaagcttcatgctctccttggcaataggtggtcgttaatagcaggaagattgccaggacgaacggataatgaagtgaagaattattggaattctcatttgacaagaaaacttataaaaatgggaattgatccaaaaaatcataggctatctcattatcttcacataaaaagacttgaattactccaagaaaataacacaagattagaaaatgttggagtaatatctgatgctacaagttcttatgctaataaagatcaacaaattacaagttcattgcttgatctcaatttaattccatag

SEQ ID NO: 16 - protein, 178 aa, Solanum lycopersicum
MRKPCCDNKEEMHKGAWSKQEDQKLIDYITKHGEGCWRNLPKAAGLLRCGKSCRLRWMNYLNPNLKRGNFSEDEDDLIIKLHALLGNRWSLIAGRLPGRTDNEVKNYWNSHLTRKLIKMGIDPKNHRLSHYLHIKRLELLQENNTRLENVGVISDATSSYANKDQQITSSLLDLNLIP

SEQ ID NO: 17 - DNA, 555 bp, Petunia axillaris
atgagaaaggcttgctgtgataacaaggaggaaatgcatagaggagcttggtctaagcaagaagaccagaagctcattgattatatcactaagcatggcgcaggttgctggcgaaatttacctaaagctgccggtctgcttcgttgcggtaaaagttgcaggctaagatggatgaattatcttagcccaaaccttaaaagaggaaatttttctgaggatgaagaggatctcatcatcaagcttcatgccctacttggcaacaggtggtctctaatagcgggtagattgccagggcgcactgataatgaagtgaagaactattggaattcccatttgagaagaaaacttataaaaatgggaattgatccaaagaatcataggatatctcattatcttcataggaaaagacttgagtattggtcagaaaatagcagcagaggaaccgatcatgaagtggtctctgatgctggaagttcttgtgcaaaacatcaaccaagttccttgcctgatctcaattcccctccttcaattcacagttcttgtgcacaaccgtag

SEQ ID NO: 18 - protein, 184 aa, Petunia axillaris
MRKACCDNKEEMHRGAWSKQEDQKLIDYITKHGAGCWRNLPKAAGLLRCGKSCRLRWMNYLSPNLKRGNFSEDEEDLIIKLHALLGNRWSLIAGRLPGRTDNEVKNYWNSHLRRKLIKMGIDPKNHRISHYLHRKRLEYWSENSSRGTDHEVVSDAGSSCAKHQPSSLPDLNSPPSIHSSCAQP